European Patent Application EP 4 442 272 A1, published October 9, 2024. Title: 一种疫苗佐剂、其制备方法及应用. Applicant: 成都迈科康生物科技有限公司. Application CN. The sequence listing filed with the application follows.

SEQUENCE LISTING (3 sequences)

SEQ ID NO: 1 - protein, 508 aa, varicella zoster virus
SVLRYDDFHTDEDKLDTNSVYEPYYHSDHAESSWVNRGESSRKAYDHNSPYIWPRNDYDGFLENAHEHHGVYNQGRGIDSGERLMQPTQMSAQEDLGDDTGIHVIPTLNGDDRHKIVNVDQRQYGDVFKGDLNPKPQGQRLIEVSVEENHPFTLRAPIQRIYGVRYTETWSFLPSLTCTGDAAPAIQHICLKHTTCFQDVVVDVDCAENTKEDQLAEISYRFQGKKEADQPWIVVNTSTLFDELELDPPEIEPGVLKVLRTEKQYLGVYIWNMRGSDGTSTYATFLVTWKGDEKTRNPTPAVTPQPRGAEFHMWNYHSHVFSVGDTFSLAMHLQYKIHEAPFDLLLEWLYVPIDPTCQPMRLYSTCLYHPNAPQCLSHMNSGCTFTSPHLAQRVASTVYQNCEHADNYTAYCLGISHMEPSFGLILHDGGTTLKFVDTPESLSGLYVFVVYFNGHVEAVAYTVVSTVDHFVNAIEERGFPPTAGQPPATTKPKEITPVNPGTSPLLRY

SEQ ID NO: 2 - protein, 268 aa, human papillomavirus
HQKRTAMFQDPQERPRKLPQLCTELQTTIHDIILECVYCKQQLLRREVYDFAFRDLCIVYRDGNPYAVGDKCLKFYSKVSEYRYYCYSLYGTTLEQQYNKPLCDLLIRGINCQKPLCPDEKQRHLDKKQRFHNIRGRWTGRCMSCCRSSRTRRETQLGSGSGSGSGSGSGMHGDTPTLHEYMLDLQPETTDLYGYGQLHDSSEEEDEIDGPAGQAEPDRAHYNIVTFCCKCDSTLRLCVQSTHVDIRTLEDLLMGTLGIVGPICSQKP

SEQ ID NO: 3 - protein, 275 aa, human papillomavirus
ARFEDPTRRPYKLPDLCTELNTSLQDIEITCVYCKTVLELTEVFEFAFKDLFVVYRDSIPHAAGHKCIDFYSRIRELRHYSDSVYGDTLEKLTNTGLYNLLIRGLRCQKPLNPAEKLRHLNEKRRFHNIAGHYRGQCHSCCNRARQERLQRRRETQVGSGSGSGSGSGSGMHGPKATLQDIVLHLEPQNEIPVDLLGHGQLSDSEEENDEIDGVNHQHLPARRAEPQRHTMLCMCCKCEARIELVVESSADDLRAFQQLFLNTLSFVGPWCASQQ